European Patent Specification EP 3 601 549 B1, published July 1, 2026. Title: POLYPEPTIDES HAVING DNASE ACTIVITY. Applicant: Novozymes A/S. The sequence listing filed with the application follows.

SEQUENCE LISTING (18 sequences)

SEQ ID NO: 1 - DNA, 645 bp, Streptomyces sp-63712
  CDS (1)..(642)
  sig_peptide (1)..(96)
  mat_peptide (97)..(642)
atggcaaaggtctacgcgcgtcgagtttccatcgccgcgggttcggccgcggccctggtctgcacgctgatgctgagcggccagaccgcccaggcagcgccgcccagcccgcccagcgcggccaccgcacggacgtacctcaccgagatcaaggagcagcccgagggcccgcaggacggctacagccgcgacaagttcccgcactggatcgaccaggggaacaactgcaacacccgcgaggtggtgctcaagcgtgatggcaccaacgtgcagcaggacggcagctgtgcggcggtcggcggcacctgggtctccgcgtacgacggcgcgacctggacccaggcgtccgacctcgacatcgaccatgtcgtaccgctgtcggaggcgtggaagtcgggcgccgcgcagtggaccaccgcgaagcgtcaggagctcgccaacgacctgacgcactcccagctgatcgccgtcaccgacaacgtcaaccaggccaagggcgacaaggacccggcgaactggctgccgccgaaggcgtcgtaccactgcgagtacgcccggatgtgggtgtgggtgaagcatgagtacggcatgaccgcggactccgcggagaaggccgccctgaagaagatcctggacggctgctga

SEQ ID NO: 2 - protein, 214 aa, Streptomyces sp-63712
MAKVYARRVSIAAGSAAALVCTLMLSGQTAQAAPPSPPSAATARTYLTEIKEQPEGPQDGYSRDKFPHWIDQGNNCNTREVVLKRDGTNVQQDGSCAAVGGTWVSAYDGATWTQASDLDIDHVVPLSEAWKSGAAQWTTAKRQELANDLTHSQLIAVTDNVNQAKGDKDPANWLPPKASYHCEYARMWVWVKHEYGMTADSAEKAALKKILDGC

SEQ ID NO: 3 - protein, 182 aa, Streptomyces sp-63712
APPSPPSAATARTYLTEIKEQPEGPQDGYSRDKFPHWIDQGNNCNTREVVLKRDGTNVQQDGSCAAVGGTWVSAYDGATWTQASDLDIDHVVPLSEAWKSGAAQWTTAKRQELANDLTHSQLIAVTDNVNQAKGDKDPANWLPPKASYHCEYARMWVWVKHEYGMTADSAEKAALKKILDGC

SEQ ID NO: 4 - DNA, 630 bp, Saccharothrix australiensis
  CDS (1)..(627)
  sig_peptide (1)..(81)
  mat_peptide (82)..(627)
ttgttacggatcagcacagccccgctcaccctgttcctgaccggcgcgctcgtcctcggcgtcgccgcgcccgcggcggccacgccgcccgacatccccggcacggccaccgcccaggccgagctggccgggctcaccgtcgccgccgagggctcgacggcgggctactcgcgcgacctgttcccgcactggaccaccgtctccggcacgtgcaacacgcgggagacggtgctcaagcgcgacggcacgtccgtggtcaccgacgcctcctgcgccgcgacgtccggccgctggtacagcccgtacgacggggccacctggagcgcggcgtccgacgtggacatcgaccacgtcgtgccgctggccgaggcgtggcggtccggcgcgtcctcgtggaccaccgcgcggcggcagtcgttcgccaacgacctcgccggaccgcagctgatcgccgtgacggacgacgtgaaccaggccaagggcgaccaggacccggcgcggtggcagccgccgctgacctcctaccggtgcacctacgccaagatgtgggtgcacaccaagcaccggtggggcctgaaggtcgactccgccgagaagtccgcgttgcagtcgatgctcgggaggtgctga

SEQ ID NO: 5 - protein, 209 aa, Saccharothrix australiensis
LLRISTAPLTLFLTGALVLGVAAPAAATPPDIPGTATAQAELAGLTVAAEGSTAGYSRDLFPHWTTVSGTCNTRETVLKRDGTSVVTDASCAATSGRWYSPYDGATWSAASDVDIDHVVPLAEAWRSGASSWTTARRQSFANDLAGPQLIAVTDDVNQAKGDQDPARWQPPLTSYRCTYAKMWVHTKHRWGLKVDSAEKSALQSMLGRC

SEQ ID NO: 6 - protein, 182 aa, Saccharothrix australiensis
TPPDIPGTATAQAELAGLTVAAEGSTAGYSRDLFPHWTTVSGTCNTRETVLKRDGTSVVTDASCAATSGRWYSPYDGATWSAASDVDIDHVVPLAEAWRSGASSWTTARRQSFANDLAGPQLIAVTDDVNQAKGDQDPARWQPPLTSYRCTYAKMWVHTKHRWGLKVDSAEKSALQSMLGRC

SEQ ID NO: 7 - DNA, 873 bp, Kutzneria albida
  CDS (1)..(636)
  sig_peptide (1)..(90)
  mat_peptide (91)..(636)
atgaatagttttcgtgccgtacgcgggctgttagccgccggagcgctgtcggtggtcgcggtcctcggggtgagcaccccggcctccgcgaccccgccgaacatcccggacaagaccaccgcggtgaacgagctcaacgggctgcgggtccagcccgacggctcctccgccggctactcgcgggacaagttcaagcactggatcaccatcgagggcagctgcaacacccgcgagatggtgctcaagcgcgacggcacgaacgtgcagaccgactcctcctgcgcggccaagtccggcacctggtacagcccgtacgacggctccacgcaaaccagcgcctcggccatccagatcgaccacatggtgccgctggccgacgcctggcgcaccggcgcctccggctggaccgcgcagcggcgccaggacttcgccaacgacctgagctacccgcagctggtggccgtcaagggcgcggtgaacgagtccaagggcgacaagtcacccgatctgtggaagcctccgctgacctcgtactggtgcacgtacgcgaagatgtggacgcacgtgaagtccaagtactcgctcactgtcaactccgcggagaagagcgctctgcaggacatgctcggtaggtgctgatggccgaatactcgtccccgttcgcgtctggccccggcggggtgatgaccgacgacgtcggggtgatcaccggcgacctcgaactgcgcaccgaggccggcgaggacggactcgtctcggtgtacgtgcgctacgaggaggcggacgagtggtaccggctgcgcggggcctcgtgcgtggtgcacgacccgcgcgaccaccgggcgctgcacatggcgctgctcggtgtgctga

SEQ ID NO: 8 - protein, 212 aa, Kutzneria albida
MNSFRAVRGLLAAGALSVVAVLGVSTPASATPPNIPDKTTAVNELNGLRVQPDGSSAGYSRDKFKHWITIEGSCNTREMVLKRDGTNVQTDSSCAAKSGTWYSPYDGSTQTSASAIQIDHMVPLADAWRTGASGWTAQRRQDFANDLSYPQLVAVKGAVNESKGDKSPDLWKPPLTSYWCTYAKMWTHVKSKYSLTVNSAEKSALQDMLGRC

SEQ ID NO: 9 - protein, 182 aa, Kutzneria albida
TPPNIPDKTTAVNELNGLRVQPDGSSAGYSRDKFKHWITIEGSCNTREMVLKRDGTNVQTDSSCAAKSGTWYSPYDGSTQTSASAIQIDHMVPLADAWRTGASGWTAQRRQDFANDLSYPQLVAVKGAVNESKGDKSPDLWKPPLTSYWCTYAKMWTHVKSKYSLTVNSAEKSALQDMLGRC

SEQ ID NO: 10 - protein, 6 aa, Artificial
  Histidine tail
HHHHHH

SEQ ID NO: 11 - protein, 5 aa, Artificial
  Motif
  MISC_FEATURE (1)..(1): X = E (Glu), D (Asp), H (His)
  MISC_FEATURE (3)..(3): X = I (Ile), V (Val), L (Leu), F (Phe), M (Met)
  misc_feature (4)..(4): Xaa can be any naturally occurring amino acid
  MISC_FEATURE (5)..(5): X = P (Pro), A (Ala), S (Ser)
XHXXX

SEQ ID NO: 12 - protein, 5 aa, Artificial
  Motif
  MISC_FEATURE (1)..(1): X= F (Phe), L (Leu), Y (Tyr), I (Ile)
  MISC_FEATURE (3)..(3): X= N (Asn), R (Arg)
  MISC_FEATURE (5)..(5): X= L (Leu), I (Ile), P (Pro), V (Val)
XAXDX

SEQ ID NO: 13 - protein, 4 aa, Artificial
  Motif
  MISC_FEATURE (2)..(2): X= D (Asp),  N (Asn)
  MISC_FEATURE (4)..(4): X= A (Ala), R (Arg)
CXTX

SEQ ID NO: 14 - protein, 4 aa, Artificial
  Motif
  MISC_FEATURE (1)..(1): X=D (Asp), Q (Gln)
  MISC_FEATURE (2)..(2): X=I (Ile), V (Val)
XXDH

SEQ ID NO: 15 - protein, 5 aa, Artificial
  Motif
  MISC_FEATURE (2)..(2): X = D (Asp), N (Asn)
CXTRE

SEQ ID NO: 16 - protein, 5 aa, Artificial
  Motif
  MISC_FEATURE (1)..(1): X= D (Asp), N (Asn)
XSAEK

SEQ ID NO: 17 - protein, 5 aa, Artificial
  Motif
  MISC_FEATURE (1)..(1): X= D (Asp), N (Asn)
  MISC_FEATURE (3)..(3): X= T (Thr), D (Asp), S (Ser), P (Pro)
XAXGY

SEQ ID NO: 18 - protein, 27 aa, bacillus clausii
MKKPLGKIVASTALLISVAFSSSIASA